European Patent Application EP 4 487 865 A1, published January 8, 2025. Title: Composition For Combi-Therapy Comprising VEGF-Grab and PD-1 or PD-L1 Antagonist. Applicant: Panolos Bioscience, Inc. The sequence listing filed with the application follows.

SEQUENCE LISTING (3 sequences)

SEQ ID NO: 1 - protein, 85 aa, synthetic construct
EFGRPFVEMYSEIPEIIHMTEGRELVIPCRVTSPNITVTLKKFPLDTLIPDGKRIIWDSRKGFIISNATYKEIGLLTCEATVNGH

SEQ ID NO: 2 - protein, 118 aa, synthetic construct
LYKTNYLTHRQTNTIIDVQISTPSPVTLLRGHTLVLNCTATTPLNTRVQMTWSYPDEKNKNASVRRRIDQSNSHANIFYSVLTIDKMQNKDKGLYTCRVRSGPSFKSVNTSVHIYDKA

SEQ ID NO: 3 - protein, 432 aa, synthetic construct
EFGRPFVEMYSEIPEIIHMTEGRELVIPCRVTSPNITVTLKKFPLDTLIPDGKRIIWDSRKGFIISNATYKEIGLLTCEATVNGHLYKTNYLTHRQTNTIIDVQISTPSPVTLLRGHTLVLNCTATTPLNTRVQMTWSYPDEKNKNASVRRRIDQSNSHANIFYSVLTIDKMQNKDKGLYTCRVRSGPSFKSVNTSVHIYDKALEDKTHTCPPCPAPELLGGPSVFLFPPKPKDTLMISRTPEVTCVVVDVSHEDPEVKFNWYVDGVEVHNAKTKPREEQYNSTYRVVSVLTVLHQDWLNGKEYKCKVSNKALPAPIEKTISKAKGQPREPQVYTLPPSREEMTKNQVSLTCLVKGFYPSDIAVEWESNGQPENNYKTTPPVLDSDGSFFLYSKLTVDKSRWQQGNVFSCSVMHEALHNHYTQKSLSLSPGK